European Patent Application EP 4 524 151 A1, published March 19, 2025. Title: Interleukin21 Variant and Fusion Protein Comprising the Same and Uses Thereof. Applicant: Ajou University Industry Academic Cooperation Foundation. The sequence listing filed with the application follows.

SEQUENCE LISTING (10 sequences)

SEQ ID NO: 1 - protein, 107 aa, synthetic construct
  REGION 1..107: note = IgG4-EW-RVT CH3A
GQPREPQVYTLPPSQEEMTENQVSLTCLVKGFYPSDIAVEWESNGQPENNYKTTPPVLDSDGSFFLYSWLTVDKSRWQEGNVFSCSVMHEALHNHYTQKSLSLSLGK

SEQ ID NO: 2 - protein, 107 aa, synthetic construct
  REGION 1..107: note = IgG4-EW-RVT CH3B
GQPREPRVYTLPPSQEEMTKNQVSLTCLVKGFYPSDIAVEWESNGQPENNYKTTPPVLVSDGSFTLYSRLTVDKSRWQEGNVFSCSVMHEALHNHYTQKSLSLSLGK

SEQ ID NO: 3 - protein, 107 aa, synthetic construct
  REGION 1..107: note = IgG4 WT
GQPREPQVYTLPPSQEEMTKNQVSLTCLVKGFYPSDIAVEWESNGQPENNYKTTPPVLDSDGSFFLYSRLTVDKSRWQEGNVFSCSVMHEALHNHYTQKSLSLSLGK

SEQ ID NO: 4 - protein, 131 aa, synthetic construct
  REGION 1..131: note = IL21
QDRHMIRMRQLIDIVDQLKNYVNDLVPEFLPAPEDVETNCEWSAFSCFQKAQLKSANTGNNERIINVSIKKLKRKPPSTNAGRRQKHRLTCPSCDSYEKKPPKEFLERFKSLLQKMIHQHLSSRTHGSEDS

SEQ ID NO: 5 - protein, 131 aa, synthetic construct
  REGION 1..131: note = IL21 NKQ
QDRHMIRMRQLIDIVDQLKNYVNDLVPEFLPAPEDVETNCEWSAFSCFQKAQLKSANTGNNERIINVSIKKLKRKPPSTNAGNKQKHRLTCPSCDSYEKKPPKEFLERFKSLLQKMIHQHLSSQTHGSEDS

SEQ ID NO: 6 - protein, 131 aa, synthetic construct
  REGION 1..131: note = IL21 DDD
QDRHMIRMRQLIDIVDQLKNYVNDLVPEFLPAPEDVETNCEWSAFSCFQKAQLKSANTGNNERIINVSIKKLKRKPPSTNAGDDQKHRLTCPSCDSYEKKPPKEFLERFKSLLQKMIHQHLSSDTHGSEDS

SEQ ID NO: 7 - protein, 131 aa, synthetic construct
  REGION 1..131: note = IL21 NQNT
QDRHMIRMRQLIDIVDQLKNYVNDLVPEFLPAPEDVETNCEWSAFSCFQNAQLQSANTGNNERIINVSIKKLKRKPPSTNAGRRQNHTLTCPSCDSYEKKPPKEFLERFKSLLQKMIHQHLSSRTHGSEDS

SEQ ID NO: 8 - protein, 131 aa, synthetic construct
  REGION 1..131: note = IL21 DDDNQNT
QDRHMIRMRQLIDIVDQLKNYVNDLVPEFLPAPEDVETNCEWSAFSCFQNAQLQSANTGNNERIINVSIKKLKRKPPSTNAGDDQNHTLTCPSCDSYEKKPPKEFLERFKSLLQKMIHQHLSSDTHGSEDS

SEQ ID NO: 9 - protein, 127 aa, synthetic construct
  REGION 1..127: note = IL21 Helix1
QDRHMIRMRQLIDIVDQLKNYVNDLVPEFLPAPEDVETNCEWSAFSCFQKAQLKSANTGNNERIINVSIKKLKRLDRNLWGLAGLTCPSCDSYEKKPPKEFLERFKSLLQKMIHQHLSSRTHGSEDS

SEQ ID NO: 10 - protein, 127 aa, synthetic construct
  REGION 1..127: note = IL21 Helix2
QDRHMIRMRQLIDIVDQLKNYVNDLVPEFLPAPEDVETNCEWSAFSCFQKAQLKSANTGNNERIINVSIKKLKRLDRNLNSLANLTCPSCDSYEKKPPKEFLERFKSLLQKMIHQHLSSRTHGSEDS